European Patent Specification EP 4 032 548 B1, published October 29, 2025. Title: COMBINED VACCINE AGAINST HUMAN RESPIRATORY SYNCYTIAL VIRUS (RSV) INFECTIONS AND METHOD THEREOF FOR INDUCING IMMUNE RESPONSE. Applicant: Beijing Jiaotong University Beijing Zhifei lvzhu Biopharmaceutical Co.,Ltd. The sequence listing filed with the application follows.

SEQUENCE LISTING (3 sequences)

SEQ ID NO: 1 - DNA, 1659 bp, Artificial Sequence
  Nucleotide sequence of Pre-fusion fusion glycoprotein
atggaactgctgatcctgaaggccaacgccatcaccaccatcctgaccgctgtgaccttctgcttcgccagcggccagaacatcaccgaggaattctaccagagcacctgtagcgccgtgtccaagggctacctgagcgccctgcggaccggctggtacaccagcgtgatcaccatcgagctgagcaacatcaagaaaatcaagtgcaacggcaccgacgccaagatcaagctgatcaagcaggaactggacaagtacaagaacgccgtgaccgagctgcagctgctgatgcagagcacccccgccaccaacaaccaggctagaggcagcggaagcggacggtccctgggcttcctgctgggcgtgggcagcgccattgctagcggagtggccgtgtcaaaggtgctgcacctggaaggcgaagtgaacaagatcaagtccgccctgctgagcaccaacaaggccgtggtgtccctgagcaacggcgtgtccgtgctgaccagcaaggtgctggatctgaagaactacatcgacaagcagctgctgcccatcgtgaacaagcagagctgcagcatccccaacatcgagacagtgatcgagttccagcagaagaacaaccggctgctggaaatcacccgcgagttcagcgtgaacgccggcgtgaccacccccgtgtccacctacatgctgaccaacagcgagctgctgagcctgatcaacgacatgcccatcaccaacgaccagaaaaagctgatgagcaacaacgtgcagatcgtgcggcagcagagctactccatcatgagcatcatcaaagaagaggtgctggcctacgtggtgcagctgcccctgtacggcgtgatcgacaccccctgctggaagctgcacaccagccccctgtgcaccaccaacaccaaagagggcagcaacatctgcctgacccggaccgaccggggctggtactgcgataatgccggcagcgtgtcattctttccacaagccgagacatgcaaggtgcagagcaaccgggtgttctgcgacaccatgaacagcctgaccctgccctccgaagtgaacctgtgcaacgtggacatcttcaaccctaagtacgactgcaagatcatgacctccaagaccgacgtgtccagctccgtgatcacctccctgggcgccatcgtgtcctgctacggcaagaccaagtgcaccgccagcaacaagaaccggggcatcatcaagaccttcagcaacggctgcgactacgtgtccaacaagggggtggacaccgtgtccgtgggcaacaccctgtactacgtgaacaaacaggaaggcaagagcctgtacgtgaagggcgagcccatcatcaacttctacgaccccctggtgttccccagcgaccagttcgacgccagcatcagccaggtcaacgagaagatcaaccagagcctggccttcatcagaaagagcgacgagctgctgcacaatgtgaatgccgtgaagtccaccaccaatatcatgatcaccacaatcatcatcgtgatcatcgtcatcctgctgtccctgatcgccgtgggcctgctgctgtactgcaaggcccggtccacccctgtgaccctgtccaaggaccagctgagcggcatcaacaatatcgccttctccaactga

SEQ ID NO: 2 - DNA, 1014 bp, Artificial Sequence
  Nucleotide sequence of attachment glycoprotein 130-230aa
atggacgccatgaagaggggcctgtgctgcgtgctgctgctgtgcggcgccgtgttcgtgagccccagcaccgtgaaaacaaagaacaccaccaccacccagacccagcccagcaagcccaccaccaagcagcggcagaacaagccccccaacaagcccaacaacgacttccacttcgaggtgttcaacttcgtgccctgcagcatctgcagcaacaaccctacctgctgggccatctgcaagcggaagcctaacaagaagcccggcaagaaaaccaccacaaagcccaccaagaagcctaccttcaagaccacaaagaaggacctgaagccccagaccaccaagcccaaagaggtgcccaccactaagcccggaggcggcggatccacagtgaaaactaagaataccacaacaacacagacacagccttccaagcctacaacaaaacagaggcagaacaaacctcctaacaaacctaacaatgattttcactttgaagtgttcaattttgtgccttgctccatctgctccaacaatccaacatgttgggctatctgtaaacgcaaacccaacaagaaacctgggaaaaagaccaccaccaaacctacaaagaaacccacctttaaaaccaccaagaaagatctgaaacctcagacaacaaaacctaaagaagtgcctactaccaagcccggaggcggcggatccaccgtgaaaacaaaaaacacaacaacaactcagactcagccctctaaacccacaactaagcagagacagaacaagcctccaaacaagccaaacaatgatttccatttcgaagtgtttaactttgtgccatgttctatctgttctaacaatcccacttgttgggccatctgcaaaagaaagccaaacaaaaaacccggcaaaaagacaacaactaagcctaccaaaaagcccacattcaaaactaccaaaaaggatctgaagccacagacaactaagccaaaagaagtgcccacaacaaaaccctgataa

SEQ ID NO: 3 - DNA, 2736 bp, Artificial Sequence
  Nucleotide sequence of Pre-fusion fusion glycoprotein and attachment glycoprotein 130-230aa
atggaactgctgatcctgaaggccaacgccatcaccaccatcctgaccgctgtgaccttctgcttcgccagcggccagaacatcaccgaggaattctaccagagcacctgtagcgccgtgtccaagggctacctgagcgccctgcggaccggctggtacaccagcgtgatcaccatcgagctgagcaacatcaagaaaatcaagtgcaacggcaccgacgccaagatcaagctgatcaagcaggaactggacaagtacaagaacgccgtgaccgagctgcagctgctgatgcagagcacccccgccaccaacaaccaggctagaggcagcggaagcggacggtccctgggcttcctgctgggcgtgggcagcgccattgctagcggagtggccgtgtcaaaggtgctgcacctggaaggcgaagtgaacaagatcaagtccgccctgctgagcaccaacaaggccgtggtgtccctgagcaacggcgtgtccgtgctgaccagcaaggtgctggatctgaagaactacatcgacaagcagctgctgcccatcgtgaacaagcagagctgcagcatccccaacatcgagacagtgatcgagttccagcagaagaacaaccggctgctggaaatcacccgcgagttcagcgtgaacgccggcgtgaccacccccgtgtccacctacatgctgaccaacagcgagctgctgagcctgatcaacgacatgcccatcaccaacgaccagaaaaagctgatgagcaacaacgtgcagatcgtgcggcagcagagctactccatcatgagcatcatcaaagaagaggtgctggcctacgtggtgcagctgcccctgtacggcgtgatcgacaccccctgctggaagctgcacaccagccccctgtgcaccaccaacaccaaagagggcagcaacatctgcctgacccggaccgaccggggctggtactgcgataatgccggcagcgtgtcattctttccacaagccgagacatgcaaggtgcagagcaaccgggtgttctgcgacaccatgaacagcctgaccctgccctccgaagtgaacctgtgcaacgtggacatcttcaaccctaagtacgactgcaagatcatgacctccaagaccgacgtgtccagctccgtgatcacctccctgggcgccatcgtgtcctgctacggcaagaccaagtgcaccgccagcaacaagaaccggggcatcatcaagaccttcagcaacggctgcgactacgtgtccaacaagggggtggacaccgtgtccgtgggcaacaccctgtactacgtgaacaaacaggaaggcaagagcctgtacgtgaagggcgagcccatcatcaacttctacgaccccctggtgttccccagcgaccagttcgacgccagcatcagccaggtcaacgagaagatcaaccagagcctggccttcatcagaaagagcgacgagctgctgcacaatgtgaatgccgtgaagtccaccaccaatatcatgatcaccacaatcatcatcgtgatcatcgtcatcctgctgtccctgatcgccgtgggcctgctgctgtactgcaaggcccggtccacccctgtgaccctgtccaaggaccagctgagcggcatcaacaatatcgccttctccaacgagggccgcggcagcctgctgacctgcggcgacgtggaggagaaccccggccccggtaccgccaccatggacgccatgaagaggggcctgtgctgcgtgctgctgctgtgcggcgccgtgttcgtgagccccagcaccgtgaaaacaaagaacaccaccaccacccagacccagcccagcaagcccaccaccaagcagcggcagaacaagccccccaacaagcccaacaacgacttccacttcgaggtgttcaacttcgtgccctgcagcatctgcagcaacaaccctacctgctgggccatctgcaagcggaagcctaacaagaagcccggcaagaaaaccaccacaaagcccaccaagaagcctaccttcaagaccacaaagaaggacctgaagccccagaccaccaagcccaaagaggtgcccaccactaagcccggaggcggcggatccacagtgaaaactaagaataccacaacaacacagacacagccttccaagcctacaacaaaacagaggcagaacaaacctcctaacaaacctaacaatgattttcactttgaagtgttcaattttgtgccttgctccatctgctccaacaatccaacatgttgggctatctgtaaacgcaaacccaacaagaaacctgggaaaaagaccaccaccaaacctacaaagaaacccacctttaaaaccaccaagaaagatctgaaacctcagacaacaaaacctaaagaagtgcctactaccaagcccggaggcggcggatccaccgtgaaaacaaaaaacacaacaacaactcagactcagccctctaaacccacaactaagcagagacagaacaagcctccaaacaagccaaacaatgatttccatttcgaagtgtttaactttgtgccatgttctatctgttctaacaatcccacttgttgggccatctgcaaaagaaagccaaacaaaaaacccggcaaaaagacaacaactaagcctaccaaaaagcccacattcaaaactaccaaaaaggatctgaagccacagacaactaagccaaaagaagtgcccacaacaaaaccctgataa